European Patent Application EP 4 756 030 A1, published June 10, 2026. Title: Method of producing immune cells. Applicant: 学校法人東京理科大学. Application JP. The sequence listing filed with the application follows.

SEQUENCE LISTING (24 sequences)

SEQ ID NO: 1 - DNA, 1311 bp, synthetic construct
  source 1..1311: mol_type = other DNA; note = ID3-ERT2 gene
  CDS 1..1311: protein_id = 2; translation = MKALSPVRGCYEAVCCLSERSLAIARGRGKGPAAEEPLSLLDDMNHCYSRLRELVPGVPRGTQLSQVEILQRVIDYILDLQVVLAEPAPGPPDGPHLPIQTAELTPELVISNDKRSFCHWDPSAGDMRAANLWPSPLMIKRSKKNSLALSLTADQMVSALLDAEPPILYSEYDPTRPFSEASMMGLLTNLADRELVHMINWAKRVPGFVDLTLHDQVHLLECAWLEILMIGLVWRSMEHPVKLLFAPNLLLDRNQGKCVEGMVEIFDMLLATSSRFRMMNLQGEEFVCLKSIILLNSGVYTFLSSTLKSLEEKDHIHRVLDKITDTLIHLMAKAGLTLQQQHQRLAQLLLILSHIRHMSNKGMEHLYSMKCKNVVPLYDLLLEAADAHRLHAPTSRGGASVEETDQSHLATAGSTSSHSLQKYYITGEAEGFPATA
atgaaggcgctgagcccggtgcgcggctgctacgaggcggtgtgctgcctgtcggaacgcagtctggccatcgcccggggccgagggaagggcccggcagctgaggagccgctgagcttgctggacgacatgaaccactgctactcccgcctgcgggaactggtacccggagtcccgagaggcactcagcttagccaggtggaaatcctacagcgcgtcatcgactacattctcgacctgcaggtagtcctggccgagccagcccctggaccccctgatggcccccaccttcccatccagacagccgagctcactccggaacttgtcatctccaacgacaaaaggagcttttgccactgggatccatctgctggagacatgagagctgccaacctttggccaagcccgctcatgatcaaacgctctaagaagaacagcctggccttgtccctgacggccgaccagatggtcagtgccttgttggatgctgagccccccatactctattccgagtatgatcctaccagacccttcagtgaagcttcgatgatgggcttactgaccaacctggcagacagggagctggttcacatgatcaactgggcgaagagggtgccaggctttgtggatttgaccctccatgatcaggtccaccttctagaatgtgcctggctagagatcctgatgattggtctcgtctggcgctccatggagcacccagtgaagctactgtttgctcctaacttgctcttggacaggaaccagggaaaatgtgtagagggcatggtggagatcttcgacatgctgctggctacatcatctcggttccgcatgatgaatctgcagggagaggagtttgtgtgcctcaaatctattattttgcttaattctggagtgtacacatttctgtccagcaccctgaagtctctggaagagaaggaccatatccaccgagtcctggacaagatcacagacactttgatccacctgatggccaaggcaggcctgaccctgcagcagcagcaccagcggctggcccagctcctcctcatcctctcccacatcaggcacatgagtaacaaaggcatggagcatctgtacagcatgaagtgcaagaacgtggtgcccctctatgacctgctgctggaggcggcggacgcccaccgcctacatgcgcccactagccgtggaggggcatccgtggaggagacggaccaaagccacttggccactgcgggctctacttcatcgcattccttgcaaaagtattacatcacgggggaggcagagggtttccctgccacagcttga

SEQ ID NO: 2 - protein, 436 aa, synthetic construct
MKALSPVRGCYEAVCCLSERSLAIARGRGKGPAAEEPLSLLDDMNHCYSRLRELVPGVPRGTQLSQVEILQRVIDYILDLQVVLAEPAPGPPDGPHLPIQTAELTPELVISNDKRSFCHWDPSAGDMRAANLWPSPLMIKRSKKNSLALSLTADQMVSALLDAEPPILYSEYDPTRPFSEASMMGLLTNLADRELVHMINWAKRVPGFVDLTLHDQVHLLECAWLEILMIGLVWRSMEHPVKLLFAPNLLLDRNQGKCVEGMVEIFDMLLATSSRFRMMNLQGEEFVCLKSIILLNSGVYTFLSSTLKSLEEKDHIHRVLDKITDTLIHLMAKAGLTLQQQHQRLAQLLLILSHIRHMSNKGMEHLYSMKCKNVVPLYDLLLEAADAHRLHAPTSRGGASVEETDQSHLATAGSTSSHSLQKYYITGEAEGFPATA

SEQ ID NO: 3 - DNA, 1524 bp, synthetic construct
  source 1..1524: mol_type = other DNA; note = hCD19-m28z-CAR gene
  CDS 1..1524: protein_id = 4; translation = MGVPTQLLGLLLLWITDAICDYKDHDGDYKDHDIDYKDDDDKDIQMTQTTSSLSASLGDRVTISCRASQDISKYLNWYQQKPDGTVKLLIYHTSRLHSGVPSRFSGSGSGTDYSLTISNLEQEDIATYFCQQGNTLPYTFGGGTKLEITGSTSGSGKPGSGEGSTKGEVKLQESGPGLVAPSQSLSVTCTVSGVSLPDYGVSWIRQPPRKGLEWLGVIWGSETTYYNSALKSRLTIIKDNSKSQVFLKMNSLQTDDTAIYYCAKHYYYGGSYAMDYWGQGTSVTVSSAAAIEFMYPPPYLDNERSNGTIIHIKEKHLCHTQSSPKLFWALVVVAGVLFCYGLLVTVALCVIWTNSRRNRLLQSDYMNMTPRRPGLTRKPYQPYAPARDFAAYRPRAKFSRSAETAANLQDPNQLYNELNLGRREEYDVLEKKRARDPEMGGKQQRRRNPQEGVYNALQKDKMAEAYSEIGTKGERRRGKGHDGLYQGLSTATKDTYDALHMQTLAPR
atgggtgtccctacccagctcctgggactgctcctgctgtggatcaccgacgccatctgcgactacaaggatcatgacggagactataaggatcacgatattgattacaaagatgacgacgacaaagacatccagatgacacagactacatcctccctgtctgcctctctgggagacagagtcaccatcagttgcagggcaagtcaggacatctctaagtatttgaattggtatcagcagaaaccagatggaactgttaaactcctgatctaccatacatcaagattacactcaggagtcccatcaaggttcagtggcagtgggtctggaacagattattctctcaccattagcaacctggagcaagaagatattgccacttacttttgccaacagggtaatacgcttccgtacacgttcggaggggggactaagttggaaataacaggctccacctctggatccggcaagcccggatctggcgagggatccaccaagggcgaggtgaaactgcaggagtcaggacctggcctggtggcgccctcacagagcctgtccgtcacatgcactgtctcaggggtctcattacccgactatggtgtaagctggattcgccagcctccacgaaagggtctggagtggctgggagtaatatggggtagtgaaaccacatactataattcagctctcaaatccagactgaccatcatcaaggacaactccaagagccaagttttcttaaaaatgaacagtctgcaaactgatgacacagccatttactactgtgccaaacattattactacggtggtagctatgctatggactactggggtcaaggaacctcagtcaccgtctcctcagcggccgcaattgagttcatgtaccctccgccttacctagacaacgagaggagcaatggaactattattcacataaaagagaaacatctttgtcatactcagtcatctcctaagctgttttgggcactggtcgtggttgctggagtcctgttttgttatggcttgctagtgacagtggctctttgtgttatctggacaaatagtagaaggaacagactccttcaaagtgactacatgaacatgactccccggaggcctgggctcactcgaaagccttaccagccctacgcccctgccagagactttgcagcgtaccgccccagagcaaaattcagcaggagtgcagagactgctgccaacctgcaggaccccaaccagctctacaatgagctcaatctagggcgaagagaggaatatgacgtcttggagaagaagcgggctcgggatccagagatgggaggcaaacagcagaggaggaggaacccccaggaaggcgtatacaatgcactgcagaaagacaagatggcagaagcctacagtgagatcggcacaaaaggcgagaggcggagaggcaaggggcacgatggcctttaccagggtctcagcactgccaccaaggacacctatgatgccctgcatatgcagaccctggcccctcgctag

SEQ ID NO: 4 - protein, 507 aa, synthetic construct
MGVPTQLLGLLLLWITDAICDYKDHDGDYKDHDIDYKDDDDKDIQMTQTTSSLSASLGDRVTISCRASQDISKYLNWYQQKPDGTVKLLIYHTSRLHSGVPSRFSGSGSGTDYSLTISNLEQEDIATYFCQQGNTLPYTFGGGTKLEITGSTSGSGKPGSGEGSTKGEVKLQESGPGLVAPSQSLSVTCTVSGVSLPDYGVSWIRQPPRKGLEWLGVIWGSETTYYNSALKSRLTIIKDNSKSQVFLKMNSLQTDDTAIYYCAKHYYYGGSYAMDYWGQGTSVTVSSAAAIEFMYPPPYLDNERSNGTIIHIKEKHLCHTQSSPKLFWALVVVAGVLFCYGLLVTVALCVIWTNSRRNRLLQSDYMNMTPRRPGLTRKPYQPYAPARDFAAYRPRAKFSRSAETAANLQDPNQLYNELNLGRREEYDVLEKKRARDPEMGGKQQRRRNPQEGVYNALQKDKMAEAYSEIGTKGERRRGKGHDGLYQGLSTATKDTYDALHMQTLAPR

SEQ ID NO: 5 - RNA, 950 nt, Homo sapiens
  source 1..950: mol_type = mRNA
  CDS 76..435: protein_id = 6; translation = MKALSPVRGCYEAVCCLSERSLAIARGRGKGPAAEEPLSLLDDMNHCYSRLRELVPGVPRGTQLSQVEILQRVIDYILDLQVVLAEPAPGPPDGPHLPIQTAELTPELVISNDKRSFCH
gcgttgcaggtcactgtagcgggacttcttttggttttctttctctttggggcacctctggactcactccccagcatgaaggcgctgagcccggtgcgcggctgctacgaggcggtgtgctgcctgtcggaacgcagtctggccatcgcccggggccgagggaagggcccggcagctgaggagccgctgagcttgctggacgacatgaaccactgctactcccgcctgcgggaactggtacccggagtcccgagaggcactcagcttagccaggtggaaatcctacagcgcgtcatcgactacattctcgacctgcaggtagtcctggccgagccagcccctggaccccctgatggcccccaccttcccatccagacagccgagctcactccggaacttgtcatctccaacgacaaaaggagcttttgccactgactcggccgtgtcctgacacctccagaacgcaggtgctggcgcccgttctgcctgggaccccgggaacctctcctgccggaagccggacggcagggatgggccccaacttcgccctgcccacttgacttcaccaaatcccttcctggagactaaacctggtgctcaggagcgaaggactgtgaacttgtggcctgaagagccagagctagctctggccaccagctgggcgacgtcaccctgctcccaccccacccccaagttctaaggtctcttcagagcgtggaggtgtggaaggagtggctgctctccaaactatgccaaggcggcggcagagctggtcttctggtctccttggagaaaggttctgttgccctgatttatgaactctataatagagtatataggttttgtaccttttttacaggaaggtgactttctgtaacaatgcgatgtatattaaactttttataaaagttaacattttgcataataaacgatttttaaacacttgtgta

SEQ ID NO: 6 - protein, 119 aa, Homo sapiens
MKALSPVRGCYEAVCCLSERSLAIARGRGKGPAAEEPLSLLDDMNHCYSRLRELVPGVPRGTQLSQVEILQRVIDYILDLQVVLAEPAPGPPDGPHLPIQTAELTPELVISNDKRSFCH

SEQ ID NO: 7 - RNA, 6327 nt, Homo sapiens
  source 1..6327: mol_type = mRNA
  CDS 232..2019: protein_id = 8
agctggcggagggcgttcgtcctgggactgcacttgctcccgtcgggtcgcccggcttcaccggacccgcaggctcccggggcagggccggggccagagctcgcgtgtcggcgggacatgcgctgcgtcgcctctaacctcgggctgtgctctttttccaggtggcccgccggtttctgagccttctgccctgcggggacacggtctgcaccctgcccgcggccacggaccatgaccatgaccctccacaccaaagcatctgggatggccctactgcatcagatccaagggaacgagctggagcccctgaaccgtccgcagctcaagatccccctggagcggcccctgggcgaggtgtacctggacagcagcaagcccgccgtgtacaactaccccgagggcgccgcctacgagttcaacgccgcggccgccgccaacgcgcaggtctacggtcagaccggcctcccctacggccccgggtctgaggctgcggcgttcggctccaacggcctggggggtttccccccactcaacagcgtgtctccgagcccgctgatgctactgcacccgccgccgcagctgtcgcctttcctgcagccccacggccagcaggtgccctactacctggagaacgagcccagcggctacacggtgcgcgaggccggcccgccggcattctacaggccaaattcagataatcgacgccagggtggcagagaaagattggccagtaccaatgacaagggaagtatggctatggaatctgccaaggagactcgctactgtgcagtgtgcaatgactatgcttcaggctaccattatggagtctggtcctgtgagggctgcaaggccttcttcaagagaagtattcaaggacataacgactatatgtgtccagccaccaaccagtgcaccattgataaaaacaggaggaagagctgccaggcctgccggctccgtaaatgctacgaagtgggaatgatgaaaggtgggatacgaaaagaccgaagaggagggagaatgttgaaacacaagcgccagagagatgatggggagggcaggggtgaagtggggtctgctggagacatgagagctgccaacctttggccaagcccgctcatgatcaaacgctctaagaagaacagcctggccttgtccctgacggccgaccagatggtcagtgccttgttggatgctgagcccccgatactctattccgagtatgatcctaccagacccttcagtgaagcttcgatgatgggcttactgaccaacctggcagacagggagctggttcacatgatcaactgggcgaagagggtgccaggctttgtggatttgaccctccatgatcaggtccaccttctagaatgtgcctggctagagatcctgatgattggtctcgtctggcgctccatggagcacccagggaagctactgtttgctcctaacttgctcttggacaggaaccagggaaaatgtgtagagggcatggtggagatcttcgacatgctgctggctacatcatctcggttccgcatgatgaatctgcagggagaggagtttgtgtgcctcaaatctattattttgcttaattctggagtgtacacatttctgtccagcaccctgaagtctctggaagagaaggaccatatccaccgagtcctggacaagatcacagacactttgatccacctgatggccaaggcaggcctgaccctgcagcagcagcaccagcggctggcccagctcctcctcatcctctcccacatcaggcacatgagtaacaaaggcatggagcatctgtacagcatgaagtgcaagaacgtggtgcccctctatgacctgctgctggagatgctggacgcccaccgcctacatgcgcccactagccgtggaggggcatccgtggaggagacggaccaaagccacttggccactgcgggctctacttcatcgcattccttgcaaaagtattacatcacgggggaggcagagggtttccctgccacggtctgagagctccctggctcccacacggttcagataatccctgctgcattttaccctcatcatgcaccactttagccaaattctgtctcctgcatacactccggcatgcatccaacaccaatggctttctagatgagtggccattcatttgcttgctcagttcttagtggcacatcttctgtcttctgttgggaacagccaaagggattccaaggctaaatctttgtaacagctctctttcccccttgctatgttactaagcgtgaggattcccgtagctcttcacagctgaactcagtctatgggttggggctcagataactctgtgcatttaagctacttgtagagacccaggcctggagagtagacattttgcctctgataagcactttttaaatggctctaagaataagccacagcaaagaatttaaagtggctcctttaattggtgacttggagaaagctaggtcaagggtttattatagcaccctcttgtattcctatggcaatgcatccttttatgaaagtggtacaccttaaagcttttatatgactgtagcagagtatctggtgattgtcaattcattccccctataggaatacaaggggcacacagggaaggcagatcccctagttggcaagactattttaacttgatacactgcagattcagatgtgctgaaagctctgcctctggctttccggtcatgggttccagttaattcatgcctcccatggacctatggagagcagcaagttgatcttagttaagtctccctatatgagggataagttcctgatttttgtttttatttttgtgttacaaaagaaagccctccctccctgaacttgcagtaaggtcagcttcaggacctgttccagtgggcactgtacttggatcttcccggcgtgtgtgtgccttacacaggggtgaactgttcactgtggtgatgcatgatgagggtaaatggtagttgaaaggagcaggggccctggtgttgcatttagccctggggcatggagctgaacagtacttgtgcaggattgttgtggctactagagaacaagagggaaagtagggcagaaactggatacagttctgaggcacagccagacttgctcagggtggccctgccacaggctgcagctacctaggaacattccttgcagaccccgcattgccctttgggggtgccctgggatccctggggtagtccagctcttcttcatttcccagcgtggccctggttggaagaagcagctgtcacagctgctgtagacagctgtgttcctacaattggcccagcaccctggggcacgggagaagggtggggaccgttgctgtcactactcaggctgactggggcctggtcagattacgtatgcccttggtggtttagagataatccaaaatcagggtttggtttggggaagaaaatcctcccccttcctcccccgccccgttccctaccgcctccactcctgccagctcatttccttcaatttcctttgacctataggctaaaaaagaaaggctcattccagccacagggcagccttccctgggcctttgcttctctagcacaattatgggttacttcctttttcttaacaaaaaagaatgtttgatttcctctgggtgaccttattgtctgtaattgaaaccctattgagaggtgatgtctgtgttagccaatgacccaggtgagctgctcgggcttctcttggtatgtcttgtttggaaaagtggatttcattcatttctgattgtccagttaagtgatcaccaaaggactgagaatctgggagggcaaaaaaaaaaaaaaagtttttatgtgcacttaaatttggggacaattttatgtatctgtgttaaggatatgtttaagaacataattcttttgttgctgtttgtttaagaagcaccttagtttgtttaagaagcaccttatatagtataatatatatttttttgaaattacattgcttgtttatcagacaattgaatgtagtaattctgttctggatttaatttgactgggttaacatgcaaaaaccaaggaaaaatatttagtttttttttttttttttgtatacttttcaagctaccttgtcatgtatacagtcatttatgcctaaagcctggtgattattcatttaaatgaagatcacatttcatatcaacttttgtatccacagtagacaaaatagcactaatccagatgcctattgttggatactgaatgacagacaatcttatgtagcaaagattatgcctgaaaaggaaaattattcagggcagctaattttgcttttaccaaaatatcagtagtaatatttttggacagtagctaatgggtcagtgggttctttttaatgtttatacttagattttcttttaaaaaaattaaaataaaacaaaaaaaaatttctaggactagacgatgtaataccagctaaagccaaacaattatacagtggaaggttttacattattcatccaatgtgtttctattcatgttaagatactactacatttgaagtgggcagagaacatcagatgattgaaatgttcgcccaggggtctccagcaactttggaaatctctttgtatttttacttgaagtgccactaatggacagcagatattttctggctgatgttggtattgggtgtaggaacatgatttaaaaaaaaactcttgcctctgctttcccccactctgaggcaagttaaaatgtaaaagatgtgatttatctggggggctcaggtatggtggggaagtggattcaggaatctggggaatggcaaatatattaagaagagtattgaaagtatttggaggaaaatggttaattctgggtgtgcaccagggttcagtagagtccacttctgccctggagaccacaaatcaactagctccatttacagccatttctaaaatggcagcttcagttctagagaagaaagaacaacatcagcagtaaagtccatggaatagctagtggtctgtgtttcttttcgccattgcctagcttgccgtaatgattctataatgccatcatgcagcaattatgagaggctaggtcatccaaagagaagaccctatcaatgtaggttgcaaaatctaacccctaaggaagtgcagtctttgatttgatttccctagtaaccttgcagatatgtttaaccaagccatagcccatgccttttgagggctgaacaaataagggacttactgataatttacttttgatcacattaaggtgttctcaccttgaaatcttatacactgaaatggccattgatttaggccactggcttagagtactccttcccctgcatgacactgattacaaatactttcctattcatactttccaattatgagatggactgtgggtactgggagtgatcactaacaccatagtaatgtctaatattcacaggcagatctgcttggggaagctagttatgtgaaaggcaaatagagtcatacagtagctcaaaaggcaaccataattctctttggtgcaggtcttgggagcgtgatctagattacactgcaccattcccaagttaatcccctgaaaacttactctcaactggagcaaatgaactttggtcccaaatatccatcttttcagtagcgttaattatgctctgtttccaactgcatttcctttccaattgaattaaagtgtggcctcgtttttagtcatttaaaattgttttctaagtaattgctgcctctattatggcacttcaattttgcactgtcttttgagattcaagaaaaatttctattcttttttttgcatccaattgtgcctgaacttttaaaatatgtaaatgctgccatgttccaaacccatcgtcagtgtgtgtgtttagagctgtgcaccctagaaacaacatattgtcccatgagcaggtgcctgagacacagacccctttgcattcacagagaggtcattggttatagagacttgaattaataagtgacattatgccagtttctgttctctcacaggtgataaacaatgctttttgtgcactacatactcttcagtgtagagctcttgttttatgggaaaaggctcaaatgccaaattgtgtttgatggattaatatgcccttttgccgatgcatactattactgatgtgactcggttttgtcgcagctttgctttgtttaatgaaacacacttgtaaacctcttttgcactttgaaaaagaatccagcgggatgctcgagcacctgtaaacaattttctcaacctatttgatgttcaaataaagaattaaactaaa

SEQ ID NO: 8 - protein, 595 aa, Homo sapiens [sequence omitted]

SEQ ID NO: 9 - RNA, 942 nt, Homo sapiens
  source 1..942: mol_type = mRNA
  CDS 1..942: protein_id = 10
gctggagacatgagagctgccaacctttggccaagcccgctcatgatcaaacgctctaagaagaacagcctggccttgtccctgacggccgaccagatggtcagtgccttgttggatgctgagcccccgatactctattccgagtatgatcctaccagacccttcagtgaagcttcgatgatgggcttactgaccaacctggcagacagggagctggttcacatgatcaactgggcgaagagggtgccaggctttgtggatttgaccctccatgatcaggtccaccttctagaatgtgcctggctagagatcctgatgattggtctcgtctggcgctccatggagcacccagggaagctactgtttgctcctaacttgctcttggacaggaaccagggaaaatgtgtagagggcatggtggagatcttcgacatgctgctggctacatcatctcggttccgcatgatgaatctgcagggagaggagtttgtgtgcctcaaatctattattttgcttaattctggagtgtacacatttctgtccagcaccctgaagtctctggaagagaaggaccatatccaccgagtcctggacaagatcacagacactttgatccacctgatggccaaggcaggcctgaccctgcagcagcagcaccagcggctggcccagctcctcctcatcctctcccacatcaggcacatgagtaacaaaggcatggagcatctgtacagcatgaagtgcaagaacgtggtgcccctctatgacctgctgctggagatgctggacgcccaccgcctacatgcgcccactagccgtggaggggcatccgtggaggagacggaccaaagccacttggccactgcgggctctacttcatcgcattccttgcaaaagtattacatcacgggggaggcagagggtttccctgccacggtctga

SEQ ID NO: 10 - protein, 313 aa, Homo sapiens
AGDMRAANLWPSPLMIKRSKKNSLALSLTADQMVSALLDAEPPILYSEYDPTRPFSEASMMGLLTNLADRELVHMINWAKRVPGFVDLTLHDQVHLLECAWLEILMIGLVWRSMEHPGKLLFAPNLLLDRNQGKCVEGMVEIFDMLLATSSRFRMMNLQGEEFVCLKSIILLNSGVYTFLSSTLKSLEEKDHIHRVLDKITDTLIHLMAKAGLTLQQQHQRLAQLLLILSHIRHMSNKGMEHLYSMKCKNVVPLYDLLLEMLDAHRLHAPTSRGGASVEETDQSHLATAGSTSSHSLQKYYITGEAEGFPATV

SEQ ID NO: 11 - DNA, 1593 bp, synthetic construct
  source 1..1593: mol_type = other DNA; note = CD19 CAR gene
  CDS 1..1593: protein_id = 12; translation = MALPVTALLLPLALLLHAARPDYKDHDGDYKDHDIDYKDDDDKDIQMTQTTSSLSASLGDRVTISCRASQDISKYLNWYQQKPDGTVKLLIYHTSRLHSGVPSRFSGSGSGTDYSLTISNLEQEDIATYFCQQGNTLPYTFGGGTKLEITGSTSGSGKPGSGEGSTKGEVKLQESGPGLVAPSQSLSVTCTVSGVSLPDYGVSWIRQPPRKGLEWLGVIWGSETTYYNSALKSRLTIIKDNSKSQVFLKMNSLQTDDTAIYYCAKHYYYGGSYAMDYWGQGTSVTVSSAAAGTTTTPAPRPPTPAPTIASQPLSLRPEACRPAAGGAVHTRGLDFACDRRPPSKPFWVLVVVGGVLACYSLLVTVAFIIFWVRKRGRKKLLYIFKQPFMRPVQTTQEEDGCSCRFPEEEEGGCELASLRVKFSRSADAPAYQQGQNQLYNELNLGRREEYDVLDKRRGRDPEMGGKPQRRKNPQEGLYNELQKDKMAEAYSEIGMKGERRRGKGHDGLYQGLSTATKDTYDALHMQALPPR
atggccttaccagtgaccgccttgctcctgccgctggccttgctgctccacgccgccaggccggactacaaggatcatgacggagactataaggatcacgatattgattacaaagatgacgacgacaaagacatccagatgacacagactacatcctccctgtctgcctctctgggagacagagtcaccatcagttgcagggcaagtcaggacatctctaagtatttgaattggtatcagcagaaaccagatggaactgttaaactcctgatctaccatacatcaagattacactcaggagtcccatcaaggttcagtggcagtgggtctggaacagattattctctcaccattagcaacctggagcaagaagatattgccacttacttttgccaacagggtaatacgcttccgtacacgttcggaggggggactaagttggaaataacaggctccacctctggatccggcaagcccggatctggcgagggatccaccaagggcgaggtgaaactgcaggagtcaggacctggcctggtggcgccctcacagagcctgtccgtcacatgcactgtctcaggggtctcattacccgactatggtgtaagctggattcgccagcctccacgaaagggtctggagtggctgggagtaatatggggtagtgaaaccacatactataattcagctctcaaatccagactgaccatcatcaaggacaactccaagagccaagttttcttaaaaatgaacagtctgcaaactgatgacacagccatttactactgtgccaaacattattactacggtggtagctatgctatggactactggggtcaaggaacctcagtcaccgtctcctcagcggccgcaggtaccaccacaacgcccgctcctcggccaccgacgccagcgccaactattgcgagtcagcctctcagtctgcgacctgaggcttgtcgaccagcagccggaggcgcagtgcacacgagggggctggacttcgcctgtgatagaagacctccttctaagcccttttgggtgctggtggtggttggtggagtcctggcttgctatagcttgctagtaacagtggcctttattattttctgggtgaggaaacggggcagaaagaaactcctgtatatattcaaacaaccatttatgagaccagtacaaactactcaagaggaagatggctgtagctgccgatttccagaagaagaagaaggaggatgtgaactggctagcctgagagtgaagttcagcaggagcgcagacgcccccgcgtaccagcagggccagaaccagctctataacgagctcaatctaggacgaagagaggagtacgatgttttggacaagagacgtggccgggaccctgagatggggggaaagccgcagagaaggaagaaccctcaggaaggcctgtacaatgaactgcagaaagataagatggcggaggcctacagtgagattgggatgaaaggcgagcgccggaggggcaaggggcacgatggcctttaccagggtctcagtacagccaccaaggacacctacgacgcccttcacatgcaggccctgccccctcgc

SEQ ID NO: 12 - protein, 531 aa, synthetic construct
MALPVTALLLPLALLLHAARPDYKDHDGDYKDHDIDYKDDDDKDIQMTQTTSSLSASLGDRVTISCRASQDISKYLNWYQQKPDGTVKLLIYHTSRLHSGVPSRFSGSGSGTDYSLTISNLEQEDIATYFCQQGNTLPYTFGGGTKLEITGSTSGSGKPGSGEGSTKGEVKLQESGPGLVAPSQSLSVTCTVSGVSLPDYGVSWIRQPPRKGLEWLGVIWGSETTYYNSALKSRLTIIKDNSKSQVFLKMNSLQTDDTAIYYCAKHYYYGGSYAMDYWGQGTSVTVSSAAAGTTTTPAPRPPTPAPTIASQPLSLRPEACRPAAGGAVHTRGLDFACDRRPPSKPFWVLVVVGGVLACYSLLVTVAFIIFWVRKRGRKKLLYIFKQPFMRPVQTTQEEDGCSCRFPEEEEGGCELASLRVKFSRSADAPAYQQGQNQLYNELNLGRREEYDVLDKRRGRDPEMGGKPQRRKNPQEGLYNELQKDKMAEAYSEIGMKGERRRGKGHDGLYQGLSTATKDTYDALHMQALPPR

SEQ ID NO: 13 - DNA, 1596 bp, synthetic construct
  source 1..1596: mol_type = other DNA; note = GD2 CAR gene
  CDS 1..1596: protein_id = 14; translation = MALPVTALLLPLALLLHAARPDYKDHDGDYKDHDIDYKDDDDKDVVMTQTPLSLPVSLGDQASISCRSSQSLVHRNGNTYLHWYLQKPGQSPKLLIHKVSNRFSGVPDRFSGSGSGTDFTLKISRVEAEDLGVYFCSQSTHVPPLTFGAGTKLELKRSTSGSGKPGSGEGSTKGEVQLLQSGPELEKPGASVMISCKASGSSFTGYNMNWVRQNIGKSLEWIGAIDPYYGGTSYNQKFKGRATLTVDKSSSTAYMHLKSLTSEDSAVYYCVSGMEYWGQGTSVTVSSAKAAAGTTTTPAPRPPTPAPTIASQPLSLRPEACRPAAGGAVHTRGLDFACDRRPPSKPFWVLVVVGGVLACYSLLVTVAFIIFWVRKRGRKKLLYIFKQPFMRPVQTTQEEDGCSCRFPEEEEGGCELASLRVKFSRSADAPAYQQGQNQLYNELNLGRREEYDVLDKRRGRDPEMGGKPQRRKNPQEGLYNELQKDKMAEAYSEIGMKGERRRGKGHDGLYQGLSTATKDTYDALHMQALPPR
atggccttaccagtgaccgccttgctcctgccgctggccttgctgctccacgccgccaggccggactacaaggatcatgacggagactataaggatcacgatattgattacaaagatgacgacgacaaagacgttgttatgacccagacacccctcagtcttcctgtaagcctgggagatcaagcgtctataagctgtaggtcttcacaaagtctcgtgcatcgaaatggcaacacttatctgcattggtacctgcaaaaaccgggacagtctcctaaacttctgattcacaaagtgagtaaccgattctctggagtacctgaccgattttctggttctggttctggtactgactttacacttaagatctccagggttgaagccgaggacctcggggtctatttctgctcacagagtacacacgtcccgccacttacgtttggtgctggaactaagctggaacttaagcgaagtacatcaggcagcggtaaacctggttctggtgagggaagcaccaagggcgaagttcagctcttgcagtcaggtccggagcttgagaaaccaggggcctccgtaatgatctcctgcaaggcttccggttccagcttcaccggctacaatatgaattgggtacgccagaatatcggcaagagtttggagtggataggcgctatcgacccgtactatgggggcacgagctataaccaaaaatttaaaggacgggcaacgctgacagttgacaagagctccagcactgcgtacatgcaccttaagagccttacatcagaggactccgcggtttattattgcgtctctggtatggaatattggggtcaagggacgtctgtaacagtctctagcgcgaaggcggccgcaggtaccaccacaacgcccgctcctcggccaccgacgccagcgccaactattgcgagtcagcctctcagtctgcgacctgaggcttgtcgaccagcagccggaggcgcagtgcacacgagggggctggacttcgcctgtgatagaagacctccttctaagcccttttgggtgctggtggtggttggtggagtcctggcttgctatagcttgctagtaacagtggcctttattattttctgggtgaggaaacggggcagaaagaaactcctgtatatattcaaacaaccatttatgagaccagtacaaactactcaagaggaagatggctgtagctgccgatttccagaagaagaagaaggaggatgtgaactggctagcctgagagtgaagttcagcaggagcgcagacgcccccgcgtaccagcagggccagaaccagctctataacgagctcaatctaggacgaagagaggagtacgatgttttggacaagagacgtggccgggaccctgagatggggggaaagccgcagagaaggaagaaccctcaggaaggcctgtacaatgaactgcagaaagataagatggcggaggcctacagtgagattgggatgaaaggcgagcgccggaggggcaaggggcacgatggcctttaccagggtctcagtacagccaccaaggacacctacgacgcccttcacatgcaggccctgccccctcgc

SEQ ID NO: 14 - protein, 532 aa, synthetic construct
MALPVTALLLPLALLLHAARPDYKDHDGDYKDHDIDYKDDDDKDVVMTQTPLSLPVSLGDQASISCRSSQSLVHRNGNTYLHWYLQKPGQSPKLLIHKVSNRFSGVPDRFSGSGSGTDFTLKISRVEAEDLGVYFCSQSTHVPPLTFGAGTKLELKRSTSGSGKPGSGEGSTKGEVQLLQSGPELEKPGASVMISCKASGSSFTGYNMNWVRQNIGKSLEWIGAIDPYYGGTSYNQKFKGRATLTVDKSSSTAYMHLKSLTSEDSAVYYCVSGMEYWGQGTSVTVSSAKAAAGTTTTPAPRPPTPAPTIASQPLSLRPEACRPAAGGAVHTRGLDFACDRRPPSKPFWVLVVVGGVLACYSLLVTVAFIIFWVRKRGRKKLLYIFKQPFMRPVQTTQEEDGCSCRFPEEEEGGCELASLRVKFSRSADAPAYQQGQNQLYNELNLGRREEYDVLDKRRGRDPEMGGKPQRRKNPQEGLYNELQKDKMAEAYSEIGMKGERRRGKGHDGLYQGLSTATKDTYDALHMQALPPR

SEQ ID NO: 15 - DNA, 2058 bp, synthetic construct
  source 1..2058: mol_type = other DNA; note = GALV-MTR
  CDS 1..2058: protein_id = 16; translation = MVLLPGSMLLTSNLHHLRHQMSPGSWKRLIILLSCVFGGGGTSLQNKNPHQPMTLTWQVLSQTGDVVWDTKAVQPPWTWWPTLKPDVCALAASLESWDIPGTDVSSSKRVRPPDSDYTAAYKQITWGAIGCSYPRARTRMASSTFYVCPRDGRTLSEARRCGGLESLYCKEWDCETTGTGYWLSKSSKDLITVKWDQNSEWTQKFQQCHQTGWCNPLKIDFTDKGKLSKDWITGKTWGLRFYVSGHPGVQFTIRLKITNMPAVAVGPDLVLVEQGPPRTSLALPPPLPPREAPPPSLPDSNSTALATSAQTPTVRKTIVTLNTPPPTTGDRLFDLVQGAFLTLNATNPGATESCWLCLAMGPPYYEAIASSGEVAYSTDLDRCRWGTQGKLTLTEVSGHGLCIGKVPFTHQHLCNQTLSINSSGDHQYLLPSNHSWWACSTGLTPCLSTSVFNQTRDFCIQVQLIPRIYYYPEEVLLQAYDNSHPRTKREAVSLTLAVLLGLGITAGIGTGSTALIKGPIDLQQGLTSLQIAIDADLRALQDSVSKLEDSLTSLSEVVLQNRRGLDLLFLKEGGLCAALKEECCFYIDHSGAVRDSMKKLKEKLDKRQLERQKSQNWYEGWFNNSPWFTTLISTIMGPLIVLLLILLFGPCILNRLVQFVKDRISVVQALVLTQQYHQLKPIEYEP
atggtattgctgcctgggtccatgcttctcacctcaaacctgcaccaccttcggcaccagatgagtcctgggagctggaaaagactgatcatcctcttaagctgcgtattcggcggcggcgggacgagtctgcaaaataagaacccccaccagcccatgaccctcacttggcaggtactgtcccaaactggagacgttgtctgggatacaaaggcagtccagcccccttggacttggtggcccacacttaaacctgatgtatgtgccttggcggctagtcttgagtcctgggatatcccgggaaccgatgtctcgtcctctaaacgagtcagacctccggactcagactatactgccgcttataagcaaatcacctggggagccatagggtgcagctaccctcgggctaggactagaatggcaagctctaccttctacgtatgtccccgggatggccggaccctttcagaagctagaaggtgcggggggctagaatccctatactgtaaagaatgggattgtgagaccacggggaccggttattggctatctaaatcctcaaaagacctcataactgtaaaatgggaccaaaatagcgaatggactcaaaaatttcaacagtgtcaccagaccggctggtgtaacccccttaaaatagatttcacagacaaaggaaaattatccaaggactggataacgggaaaaacctggggattaagattctatgtgtctggacatccaggcgtacagttcaccattcgcttaaaaatcaccaacatgccagctgtggcagtaggtcctgacctcgtccttgtggaacaaggacctcctagaacgtccctcgctctcccacctcctcttcccccaagggaagcgccaccgccatctctccccgactctaactccacagccctggcgactagtgcacaaactcccacggtgagaaaaacaattgttaccctaaacactccgcctcccaccacaggcgacagactttttgatcttgtgcagggggccttcctaaccttaaatgctaccaacccaggggccactgagtcttgctggctttgtttggccatgggccccccttattatgaagcaatagcctcatcaggagaggtcgcctactccaccgaccttgaccggtgccgctgggggacccaaggaaagctcaccctcactgaggtctcaggacacgggttgtgcataggaaaggtgccctttacccatcagcatctctgcaatcagaccctatccatcaattcctccggagaccatcagtatctgctcccctccaaccatagctggtgggcttgcagcactggcctcaccccttgcctctccacctcagtttttaatcagactagagatttctgtatccaggtccagctgattcctcgcatctattactatcctgaagaagttttgttacaggcctatgacaattctcaccccaggactaaaagagaggctgtctcacttaccctagctgttttactggggttgggaatcacggcgggaataggtactggttcaactgccttaattaaaggacctatagacctccagcaaggcctgacaagcctccagatcgccatagatgctgacctccgggccctccaagactcagtcagcaagttagaggactcactgacttccctgtccgaggtagtgctccaaaataggagaggccttgacttgctgtttctaaaagaaggtggcctctgtgcggccctaaaggaagagtgctgtttttacatagaccactcaggtgcagtacgggactccatgaaaaaactcaaagaaaaactggataaaagacagttagagcgccagaaaagccaaaactggtatgaaggatggttcaataactccccttggtttaccaccttgatatctaccattatgggacccctcattgtactcctattgattttgctcttcggaccctgcattcttaatcgattagtccaatttgttaaagacaggatatcagtggtccaggctctagttttgactcaacaatatcaccagctgaagcctatagagtacgagcca

SEQ ID NO: 16 - protein, 686 aa, synthetic construct
MVLLPGSMLLTSNLHHLRHQMSPGSWKRLIILLSCVFGGGGTSLQNKNPHQPMTLTWQVLSQTGDVVWDTKAVQPPWTWWPTLKPDVCALAASLESWDIPGTDVSSSKRVRPPDSDYTAAYKQITWGAIGCSYPRARTRMASSTFYVCPRDGRTLSEARRCGGLESLYCKEWDCETTGTGYWLSKSSKDLITVKWDQNSEWTQKFQQCHQTGWCNPLKIDFTDKGKLSKDWITGKTWGLRFYVSGHPGVQFTIRLKITNMPAVAVGPDLVLVEQGPPRTSLALPPPLPPREAPPPSLPDSNSTALATSAQTPTVRKTIVTLNTPPPTTGDRLFDLVQGAFLTLNATNPGATESCWLCLAMGPPYYEAIASSGEVAYSTDLDRCRWGTQGKLTLTEVSGHGLCIGKVPFTHQHLCNQTLSINSSGDHQYLLPSNHSWWACSTGLTPCLSTSVFNQTRDFCIQVQLIPRIYYYPEEVLLQAYDNSHPRTKREAVSLTLAVLLGLGITAGIGTGSTALIKGPIDLQQGLTSLQIAIDADLRALQDSVSKLEDSLTSLSEVVLQNRRGLDLLFLKEGGLCAALKEECCFYIDHSGAVRDSMKKLKEKLDKRQLERQKSQNWYEGWFNNSPWFTTLISTIMGPLIVLLLILLFGPCILNRLVQFVKDRISVVQALVLTQQYHQLKPIEYEP

SEQ ID NO: 17 - DNA, 1821 bp, synthetic construct
  source 1..1821: mol_type = other DNA; note = OTI-TCR gene
  CDS 1..1821: protein_id = 18; translation = MDKILTASFLLLGLHLAGVNGQQQEKRDQQQVRQSPQSLTVWEGETAILNCSYEDSTFNYFPWYQQFPGEGPALLISIRSVSDKKEDGRFTIFFNKREKKLSLHITDSQPGDSATYFCAASDNYQLIWGSGTKLIIKPDIQNPEPAVYQLKDPRSQDSTLCLFTDFDSQINVPKTMESGTFITDKTVLDMKAMDSKSNGAIAWSNQTSFTCQDIFKETNATYPSSDVPCDATLTEKSFETDMNLNFQNLSVMGLRILLLKVAGFNLLMTLRLWSSGEGRGSLLTCGDVEENPGPMSNTVLADSAWGITLLSWVTVFLLGTSSADSGVVQSPRHIIKEKGGRSVLTCIPISGHSNVVWYQQTLGKELKFLIQHYEKVERDKGFLPSRFSVQQFDDYHSEMNMSALELEDSAMYFCASSRANYEQYFGPGTRLTVLEDLRNVTPPKVSLFEPSKAEIANKQKATLVCLARGFFPDHVELSWWVNGKEVHSGVSTDPQAYKESNYSYCLSSRLRVSATFWHNPRNHFRCQVQFHGLSEEDKWPEGSPKPVTQNISAEAWGRADCGITSASYHQGVLSATILYEILLGKATLYAVLVSGLVLMAMVKKKNS
atggacaagatcctgacagcatcgtttttactcctaggccttcacctagctggggtgaatggccagcagcaggagaaacgtgaccagcagcaggtgagacaaagtccccaatctctgacagtctgggaaggagagaccgcaattctgaactgcagttatgaggacagcacttttaactacttcccatggtaccagcagttccctggggaaggccctgcactcctgatatccatacgttcagtgtccgataaaaaggaagatggacgattcacaatcttcttcaataaaagggagaaaaagctctccttgcacatcacagactctcagcctggagactcagctacctacttctgtgcagcaagtgacaactatcagttgatctggggctctgggaccaagctaattataaagccagacatccagaacccagaacctgctgtgtaccagttaaaagatcctcggtctcaggacagcaccctctgcctgttcaccgactttgactcccaaatcaatgtgccgaaaaccatggaatctggaacgttcatcactgacaaaactgtgctggacatgaaagctatggattccaagagcaatggggccattgcctggagcaaccagacaagcttcacctgccaagatatcttcaaagagaccaacgccacctaccccagttcagacgttccctgtgatgccacgttgactgagaaaagctttgaaacagatatgaacctaaactttcaaaacctgtcagttatgggactccgaatcctcctgctgaaagtagccggatttaacctgctcatgacgctgaggctgtggtcctccggagagggcagaggaagtctgctaacatgcggtgacgtcgaggagaatcctggcccaatgtctaacactgtcctcgctgattctgcctggggcatcaccctgctatcttgggttactgtctttctcttgggaacaagttcagcagattctggggttgtccagtctccaagacacataatcaaagaaaagggaggaaggtccgttctgacgtgtattcccatctctggacatagcaatgtggtctggtaccagcagactctggggaaggaattaaagttccttattcagcattatgaaaaggtggagagagacaaaggattcctacccagcagattctcagtccaacagtttgatgactatcactctgaaatgaacatgagtgccttggaactggaggactctgctatgtacttctgtgccagctctcgggccaattatgaacagtacttcggtcccggcaccaggctcacggttttagaggatctgagaaatgtgactccacccaaggtctccttgtttgagccatcaaaagcagagattgcaaacaaacaaaaggctaccctcgtgtgcttggccaggggcttcttccctgaccacgtggagctgagctggtgggtgaatggcaaggaggtccacagtggggtcagcacggaccctcaggcctacaaggagagcaattatagctactgcctgagcagccgcctgagggtctctgctaccttctggcacaatcctcgaaaccacttccgctgccaagtgcagttccatgggctttcagaggaggacaagtggccagagggctcacccaaacctgtcacacagaacatcagtgcagaggcctggggccgagcagactgtggaatcacttcagcatcctatcatcagggggttctgtctgcaaccatcctctatgagatcctactggggaaggccaccctatatgctgtgctggtcagtggcctggtgctgatggccatggtcaagaaaaaaaattcc

SEQ ID NO: 18 - protein, 607 aa, synthetic construct
MDKILTASFLLLGLHLAGVNGQQQEKRDQQQVRQSPQSLTVWEGETAILNCSYEDSTFNYFPWYQQFPGEGPALLISIRSVSDKKEDGRFTIFFNKREKKLSLHITDSQPGDSATYFCAASDNYQLIWGSGTKLIIKPDIQNPEPAVYQLKDPRSQDSTLCLFTDFDSQINVPKTMESGTFITDKTVLDMKAMDSKSNGAIAWSNQTSFTCQDIFKETNATYPSSDVPCDATLTEKSFETDMNLNFQNLSVMGLRILLLKVAGFNLLMTLRLWSSGEGRGSLLTCGDVEENPGPMSNTVLADSAWGITLLSWVTVFLLGTSSADSGVVQSPRHIIKEKGGRSVLTCIPISGHSNVVWYQQTLGKELKFLIQHYEKVERDKGFLPSRFSVQQFDDYHSEMNMSALELEDSAMYFCASSRANYEQYFGPGTRLTVLEDLRNVTPPKVSLFEPSKAEIANKQKATLVCLARGFFPDHVELSWWVNGKEVHSGVSTDPQAYKESNYSYCLSSRLRVSATFWHNPRNHFRCQVQFHGLSEEDKWPEGSPKPVTQNISAEAWGRADCGITSASYHQGVLSATILYEILLGKATLYAVLVSGLVLMAMVKKKNS

SEQ ID NO: 19 - RNA, 3779 nt, Homo sapiens
  source 1..3779: mol_type = mRNA
  CDS 940..3111: protein_id = 20; translation = MGSRCALALAVLSALLCQVWSSGVFELKLQEFVNKKGLLGNRNCCRGGAGPPPCACRTFFRVCLKHYQASVSPEPPCTYGSAVTPVLGVDSFSLPDGGGADSAFSNPIRFPFGFTWPGTFSLIIEALHTDSPDDLATENPERLISRLATQRHLTVGEEWSQDLHSSGRTDLKYSYRFVCDEHYYGEGCSVFCRPRDDAFGHFTCGERGEKVCNPGWKGPYCTEPICLPGCDEQHGFCDKPGECKCRVGWQGRYCDECIRYPGCLHGTCQQPWQCNCQEGWGGLFCNQDLNYCTHHKPCKNGATCTNTGQGSYTCSCRPGYTGATCELGIDECDPSPCKNGGSCTDLENSYSCTCPPGFYGKICELSAMTCADGPCFNGGRCSDSPDGGYSCRCPVGYSGFNCEKKIDYCSSSPCSNGAKCVDLGDAYLCRCQAGFSGRHCDDNVDDCASSPCANGGTCRDGVNDFSCTCPPGYTGRNCSAPVSRCEHAPCHNGATCHERGHRYVCECARGYGGPNCQFLLPELPPGPAVVDLTEKLEGQGGPFPWVAVCAGVILVLMLLLGCAAVVVCVRLRLQKHRPPADPCRGETETMNNLANCQREKDISVSIIGATQIKNTNKKADFHGDHSADKNGFKARYPAVDYNLVQDLKGDDTAVRDAHSKRDTKCQPQGSSGEEKGTPTTLRGGEASERKRPDSGCSTSKDTKYQSVYVISEEKDECVIATEV
actgaccatttggcgatccattgagaggagggtttggaaaagtggctcctttgtgacagctctcgccagattggggggctgctgatttgcatctcattagccatgcgggcggccggctgaatataagggcggcaggcgccggcgagagccagatcctctgcgcgcacccgcggagacccgacccggccgagggcagagcgcaggggaacccgggcagccgcggcgcagagcctcctcccacggcccggcccctccggtcctgcgcgtgtgtactggatggcattggctggattcatcggaaagacgcggatctttgctgtgacaccggagatcggagcccggagtgctcccggaacgaccgccgccgccgagtgacaccgggccgcgatccgcaggggccgccgcgcacacccgccgccgccgaccgtcccctcagcgcgcgccgctggccccggattatcgccttgcccgtgggatttccagaccgcggctttctaatcggctcgggaggaagctctgcagctctcttgggaattaagctcaatctctggactctctctctttctctttctccccctccctctcctgcgaagaagctcaagacaaaaccaggaagccggcgaccctcacctcctcgggggctgggaggaaggaggaaaacgaaagtcgccgccgccgcgctgtcccccgagagctgcctttcctcgggcatccctggggctgccgcgggacctcgcagggcggatataaagaaccgcggccttgggaagaggcggagaccggcttttaaagaaagaagtcctgggtcctgcggtctggggcgaggcaagggcgcttttctgcccacgctccccgtggcccatcgatcccccgcgcgtccgccgctgttctaaggagagaagtgggggccccccaggctcgcgcgtggagcgaagcagcatgggcagtcggtgcgcgctggccctggcggtgctctcggccttgctgtgtcaggtctggagctctggggtgttcgaactgaagctgcaggagttcgtcaacaagaaggggctgctggggaaccgcaactgctgccgcgggggcgcggggccaccgccgtgcgcctgccggaccttcttccgcgtgtgcctcaagcactaccaggccagcgtgtcccccgagccgccctgcacctacggcagcgccgtcacccccgtgctgggcgtcgactccttcagtctgcccgacggcgggggcgccgactccgcgttcagcaaccccatccgcttccccttcggcttcacctggccgggcaccttctctctgattattgaagctctccacacagattctcctgatgacctcgcaacagaaaacccagaaagactcatcagccgcctggccacccagaggcacctgacggtgggcgaggagtggtcccaggacctgcacagcagcggccgcacggacctcaagtactcctaccgcttcgtgtgtgacgaacactactacggagagggctgctccgttttctgccgtccccgggacgatgccttcggccacttcacctgtggggagcgtggggagaaagtgtgcaaccctggctggaaagggccctactgcacagagccgatctgcctgcctggatgtgatgagcagcatggattttgtgacaaaccaggggaatgcaagtgcagagtgggctggcagggccggtactgtgacgagtgtatccgctatccaggctgtctccatggcacctgccagcagccctggcagtgcaactgccaggaaggctgggggggccttttctgcaaccaggacctgaactactgcacacaccataagccctgcaagaatggagccacctgcaccaacacgggccaggggagctacacttgctcttgccggcctgggtacacaggtgccacctgcgagctggggattgacgagtgtgaccccagcccttgtaagaacggagggagctgcacggatctcgagaacagctactcctgtacctgcccacccggcttctacggcaaaatctgtgaattgagtgccatgacctgtgcggacggcccttgctttaacgggggtcggtgctcagacagccccgatggagggtacagctgccgctgccccgtgggctactccggcttcaactgtgagaagaaaattgactactgcagctcttcaccctgttctaatggtgccaagtgtgtggacctcggtgatgcctacctgtgccgctgccaggccggcttctcggggaggcactgtgacgacaacgtggacgactgcgcctcctccccgtgcgccaacgggggcacctgccgggatggcgtgaacgacttctcctgcacctgcccgcctggctacacgggcaggaactgcagtgcccccgtcagcaggtgcgagcacgcaccctgccacaatggggccacctgccacgagaggggccaccgctatgtgtgcgagtgtgcccgaggctacgggggtcccaactgccagttcctgctccccgagctgcccccgggcccagcggtggtggacctcactgagaagctagagggccagggcgggccattcccctgggtggccgtgtgcgccggggtcatccttgtcctcatgctgctgctgggctgtgccgctgtggtggtctgcgtccggctgaggctgcagaagcaccggcccccagccgacccctgccggggggagacggagaccatgaacaacctggccaactgccagcgtgagaaggacatctcagtcagcatcatcggggccacgcagatcaagaacaccaacaagaaggcggacttccacggggaccacagcgccgacaagaatggcttcaaggcccgctacccagcggtggactataacctcgtgcaggacctcaagggtgacgacaccgccgtcagggacgcgcacagcaagcgtgacaccaagtgccagccccagggctcctcaggggaggagaaggggaccccgaccacactcaggggtggagaagcatctgaaagaaaaaggccggactcgggctgttcaacttcaaaagacaccaagtaccagtcggtgtacgtcatatccgaggagaaggatgagtgcgtcatagcaactgaggtgtaaaatggaagtgagatggcaagactcccgtttctcttaaaataagtaaaattccaaggatatatgccccaacgaatgctgctgaagaggagggaggcctcgtggactgctgctgagaaaccgagttcagaccgagcaggttctcctcctgaggtcctcgacgcctgccgacagcctgtcgcggcccggccgcctgcggcactgccttccgtgacgtcgccgttgcactatggacagttgctcttaagagaatatatatttaaatgggtgaactgaattacgcataagaagcatgcactgcctgagtgtatattttggattcttatgagccagtcttttcttgaattagaaacacaaacactgcctttattgtcctttttgatacgaagatgtgctttttctagatggaaaagatgtgtgttattttttggatttgtaaaaatatttttcatgatatctgtaaagcttgagtattttgtgatgttcgttttttataatttaaattttggtaaatatgtacaaaggcacttcgggtctatgtgactatatttttttgtatataaatgtatttatggaatattgtgcaaatgttatttgagttttttactgttttgttaatgaagaaattcctttttaaaatatttttccaaaataaattttatgaatgacaa

SEQ ID NO: 20 - protein, 723 aa, Homo sapiens
MGSRCALALAVLSALLCQVWSSGVFELKLQEFVNKKGLLGNRNCCRGGAGPPPCACRTFFRVCLKHYQASVSPEPPCTYGSAVTPVLGVDSFSLPDGGGADSAFSNPIRFPFGFTWPGTFSLIIEALHTDSPDDLATENPERLISRLATQRHLTVGEEWSQDLHSSGRTDLKYSYRFVCDEHYYGEGCSVFCRPRDDAFGHFTCGERGEKVCNPGWKGPYCTEPICLPGCDEQHGFCDKPGECKCRVGWQGRYCDECIRYPGCLHGTCQQPWQCNCQEGWGGLFCNQDLNYCTHHKPCKNGATCTNTGQGSYTCSCRPGYTGATCELGIDECDPSPCKNGGSCTDLENSYSCTCPPGFYGKICELSAMTCADGPCFNGGRCSDSPDGGYSCRCPVGYSGFNCEKKIDYCSSSPCSNGAKCVDLGDAYLCRCQAGFSGRHCDDNVDDCASSPCANGGTCRDGVNDFSCTCPPGYTGRNCSAPVSRCEHAPCHNGATCHERGHRYVCECARGYGGPNCQFLLPELPPGPAVVDLTEKLEGQGGPFPWVAVCAGVILVLMLLLGCAAVVVCVRLRLQKHRPPADPCRGETETMNNLANCQREKDISVSIIGATQIKNTNKKADFHGDHSADKNGFKARYPAVDYNLVQDLKGDDTAVRDAHSKRDTKCQPQGSSGEEKGTPTTLRGGEASERKRPDSGCSTSKDTKYQSVYVISEEKDECVIATEV

SEQ ID NO: 21 - RNA, 3426 nt, Homo sapiens
  source 1..3426: mol_type = mRNA
  CDS 330..2387: protein_id = 22; translation = MAAASRSASGWALLLLVALWQQRAAGSGVFQLQLQEFINERGVLASGRPCEPGCRTFFRVCLKHFQAVVSPGPCTFGTVSTPVLGTNSFAVRDDSSGGGRNPLQLPFNFTWPGTFSLIIEAWHAPGDDLRPEALPPDALISKIAIQGSLAVGQNWLLDEQTSTLTRLRYSYRVICSDNYYGDNCSRLCKKRNDHFGHYVCQPDGNLSCLPGWTGEYCQQPICLSGCHEQNGYCSKPAECLCRPGWQGRLCNECIPHNGCRHGTCSTPWQCTCDEGWGGLFCDQDLNYCTHHSPCKNGATCSNSGQRSYTCTCRPGYTGVDCELELSECDSNPCRNGGSCKDQEDGYHCLCPPGYYGLHCEHSTLSCADSPCFNGGSCRERNQGANYACECPPNFTGSNCEKKVDRCTSNPCANGGQCLNRGPSRMCRCRPGFTGTYCELHVSDCARNPCAHGGTCHDLENGLMCTCPAGFSGRRCEVRTSIDACASSPCFNRATCYTDLSTDTFVCNCPYGFVGSRCEFPVGLPPSFPWVAVSLGVGLAVLLVLLGMVAVAVRQLRLRRPDDGSREAMNNLSDFQKDNLIPAAQLKNTNQKKELEVDCGLDKSNCGKQQNHTLDYNLAPGPLGRGTMPGKFPHSDKSLGEKAPLRLHSEKPECRISAICSPRDSMYQSVCLISEERNECVIATEV
agtagcggcgctgcgcgcaggccgggaacacgaggccaagagccgcagccccagccgccttggtgcagcgtacaccggcactagcccgcttgcagccccaggattagacagaagacgcgtcctcggcgcggtcgccgcccagccgtagtcacctggattacctacagcggcagctgcagcggagccagcgagaaggccaaaggggagcagcgtcccgagaggagcgcctcttttcagggaccccgccggctggcggacgcgcgggaaagcggcgtcgcgaacagagccagattgagggcccgcgggtggagagagcgacgcccgaggggatggcggcagcgtcccggagcgcctctggctgggcgctactgctgctggtggcactttggcagcagcgcgcggccggctccggcgtcttccagctgcagctgcaggagttcatcaacgagcgcggcgtactggccagtgggcggccttgcgagcccggctgccggactttcttccgcgtctgccttaagcacttccaggcggtcgtctcgcccggaccctgcaccttcgggaccgtctccacgccggtattgggcaccaactccttcgctgtccgggacgacagtagcggcggggggcgcaaccctctccaactgcccttcaatttcacctggccgggtaccttctcgctcatcatcgaagcttggcacgcgccaggagacgacctgcggccagaggccttgccaccagatgcactcatcagcaagatcgccatccagggctccctagctgtgggtcagaactggttattggatgagcaaaccagcaccctcacaaggctgcgctactcttaccgggtcatctgcagtgacaactactatggagacaactgctcccgcctgtgcaagaagcgcaatgaccacttcggccactatgtgtgccagccagatggcaacttgtcctgcctgcccggttggactggggaatattgccaacagcctatctgtctttcgggctgtcatgaacagaatggctactgcagcaagccagcagagtgcctctgccgcccaggctggcagggccggctgtgtaacgaatgcatcccccacaatggctgtcgccacggcacctgcagcactccctggcaatgtacttgtgatgagggctggggaggcctgttttgtgaccaagatctcaactactgcacccaccactccccatgcaagaatggggcaacgtgctccaacagtgggcagcgaagctacacctgcacctgtcgcccaggctacactggtgtggactgtgagctggagctcagcgagtgtgacagcaacccctgtcgcaatggaggcagctgtaaggaccaggaggatggctaccactgcctgtgtcctccgggctactatggcctgcattgtgaacacagcaccttgagctgcgccgactccccctgcttcaatgggggctcctgccgggagcgcaaccagggggccaactatgcttgtgaatgtccccccaacttcaccggctccaactgcgagaagaaagtggacaggtgcaccagcaacccctgtgccaacgggggacagtgcctgaaccgaggtccaagccgcatgtgccgctgccgtcctggattcacgggcacctactgtgaactccacgtcagcgactgtgcccgtaacccttgcgcccacggtggcacttgccatgacctggagaatgggctcatgtgcacctgccctgccggcttctctggccgacgctgtgaggtgcggacatccatcgatgcctgtgcctcgagtccctgcttcaacagggccacctgctacaccgacctctccacagacacctttgtgtgcaactgcccttatggctttgtgggcagccgctgcgagttccccgtgggcttgccgcccagcttcccctgggtggccgtctcgctgggtgtggggctggcagtgctgctggtactgctgggcatggtggcagtggctgtgcggcagctgcggcttcgacggccggacgacggcagcagggaagccatgaacaacttgtcggacttccagaaggacaacctgattcctgccgcccagcttaaaaacacaaaccagaagaaggagctggaagtggactgtggcctggacaagtccaactgtggcaaacagcaaaaccacacattggactataatctggccccagggcccctggggcgggggaccatgccaggaaagtttccccacagtgacaagagcttaggagagaaggcgccactgcggttacacagtgaaaagccagagtgtcggatatcagcgatatgctcccccagggactccatgtaccagtctgtgtgtttgatatcagaggagaggaatgaatgtgtcattgccacggaggtataaggcaggagcctacctggacatccctgctcagccccgcggctggaccttccttctgcattgtttacattgcatcctggatgggacgtttttcatatgcaacgtgctgctctcaggaggaggagggaatggcaggaaccggacagactgtgaacttgccaagagatgcaatacccttccacacctttgggtgtctgtctggcatcagattggcagctgcaccaaccagaggaacagaagagaagagagatgccactgggcactgccctgccagtagtggccttcagggggctccttccggggctccggcctgttttccagagagagtggcagtagccccatggggcccggagctgctgtggcctccactggcatccgtgtttccaaaagtgcctttggcccaggctccacggcgacagttgggcccaaatcagaaaggagagagggggccaatgagggcagggcctcctgtgggctggaaaaccactgggtgcgtctcttgctggggtttgccctggaggtgaggtgagtgctcgagggaggggagtgctttctgccccatgcctccaactactgtatgcaggcctggctctctggtctaggccctttgggcaagaatgtccgtctacccggcttccaccaccctctggccctgggcttctgtaagcagacaggcagagggcctgcccctcccaccagccaagggtgccaggcctaactggggcactcagggcagtgtgttggaaattccactgagggggaaatcaggtgctgcggccgcctgggccctttcctccctcaagcccatctccacaacctcgagcctgggctctggtccactactgccccagaccaccctcaaagctggtcttcagaaatcaataatatgagtttttattttgtttttttttttttttttgtagtttattttggagtctagtatttcaataatttaagaatcagaagcactgacctttctacattttataacattattttgtatataatgtgtatttataatatgaaacagatgtgtacagga

SEQ ID NO: 22 - protein, 685 aa, Homo sapiens
MAAASRSASGWALLLLVALWQQRAAGSGVFQLQLQEFINERGVLASGRPCEPGCRTFFRVCLKHFQAVVSPGPCTFGTVSTPVLGTNSFAVRDDSSGGGRNPLQLPFNFTWPGTFSLIIEAWHAPGDDLRPEALPPDALISKIAIQGSLAVGQNWLLDEQTSTLTRLRYSYRVICSDNYYGDNCSRLCKKRNDHFGHYVCQPDGNLSCLPGWTGEYCQQPICLSGCHEQNGYCSKPAECLCRPGWQGRLCNECIPHNGCRHGTCSTPWQCTCDEGWGGLFCDQDLNYCTHHSPCKNGATCSNSGQRSYTCTCRPGYTGVDCELELSECDSNPCRNGGSCKDQEDGYHCLCPPGYYGLHCEHSTLSCADSPCFNGGSCRERNQGANYACECPPNFTGSNCEKKVDRCTSNPCANGGQCLNRGPSRMCRCRPGFTGTYCELHVSDCARNPCAHGGTCHDLENGLMCTCPAGFSGRRCEVRTSIDACASSPCFNRATCYTDLSTDTFVCNCPYGFVGSRCEFPVGLPPSFPWVAVSLGVGLAVLLVLLGMVAVAVRQLRLRRPDDGSREAMNNLSDFQKDNLIPAAQLKNTNQKKELEVDCGLDKSNCGKQQNHTLDYNLAPGPLGRGTMPGKFPHSDKSLGEKAPLRLHSEKPECRISAICSPRDSMYQSVCLISEERNECVIATEV

SEQ ID NO: 23 - RNA, 2058 nt, Gibbon ape leukemia virus
  source 1..2058: mol_type = mRNA
  CDS 1..2058: protein_id = 24; translation = MVLLPGSMLLTSNLHHLRHQMSPGSWKRLIILLSCVFGGGGTSLQNKNPHQPMTLTWQVLSQTGDVVWDTKAVQPPWTWWPTLKPDVCALAASLESWDIPGTDVSSSKRVRPPDSDYTAAYKQITWGAIGCSYPRARTRMASSTFYVCPRDGRTLSEARRCGGLESLYCKEWDCETTGTGYWLSKSSKDLITVKWDQNSEWTQKFQQCHQTGWCNPLKIDFTDKGKLSKDWITGKTWGLRFYVSGHPGVQFTIRLKITNMPAVAVGPDLVLVEQGPPRTSLALPPPLPPREAPPPSLPDSNSTALATSAQTPTVRKTIVTLNTPPPTTGDRLFDLVQGAFLTLNATNPGATESCWLCLAMGPPYYEAIASSGEVAYSTDLDRCRWGTQGKLTLTEVSGHGLCIGKVPFTHQHLCNQTLSINSSGDHQYLLPSNHSWWACSTGLTPCLSTSVFNQTRDFCIQVQLIPRIYYYPEEVLLQAYDNSHPRTKREAVSLTLAVLLGLGITAGIGTGSTALIKGPIDLQQGLTSLQIAIDADLRALQDSVSKLEDSLTSLSEVVLQNRRGLDLLFLKEGGLCAALKEECCFYIDHSGAVRDSMKKLKEKLDKRQLERQKSQNWYEGWFNNSPWFTTLLSTIAGPLLLLLLLLILGPCIINKLVQFINDRISAVKILVLRQKYQALENEGNL
atggtattgctgcctgggtccatgcttctcacctcaaacctgcaccaccttcggcaccagatgagtcctgggagctggaaaagactgatcatcctcttaagctgcgtattcggcggcggcgggacgagtctgcaaaataagaacccccaccagcccatgaccctcacttggcaggtactgtcccaaactggagacgttgtctgggatacaaaggcagtccagcccccttggacttggtggcccacacttaaacctgatgtatgtgccttggcggctagtcttgagtcctgggatatcccgggaaccgatgtctcgtcctctaaacgagtcagacctccggactcagactatactgccgcttataagcaaatcacctggggagccatagggtgcagctaccctcgggctaggactagaatggcaagctctaccttctacgtatgtccccgggatggccggaccctttcagaagctagaaggtgcggggggctagaatccctatactgtaaagaatgggattgtgagaccacggggaccggttattggctatctaaatcctcaaaagacctcataactgtaaaatgggaccaaaatagcgaatggactcaaaaatttcaacagtgtcaccagaccggctggtgtaacccccttaaaatagatttcacagacaaaggaaaattatccaaggactggataacgggaaaaacctggggattaagattctatgtgtctggacatccaggcgtacagttcaccattcgcttaaaaatcaccaacatgccagctgtggcagtaggtcctgacctcgtccttgtggaacaaggacctcctagaacgtccctcgctctcccacctcctcttcccccaagggaagcgccaccgccatctctccccgactctaactccacagccctggcgactagtgcacaaactcccacggtgagaaaaacaattgttaccctaaacactccgcctcccaccacaggcgacagactttttgatcttgtgcagggggccttcctaaccttaaatgctaccaacccaggggccactgagtcttgctggctttgtttggccatgggccccccttattatgaagcaatagcctcatcaggagaggtcgcctactccaccgaccttgaccggtgccgctgggggacccaaggaaagctcaccctcactgaggtctcaggacacgggttgtgcataggaaaggtgccctttacccatcagcatctctgcaatcagaccctatccatcaattcctccggagaccatcagtatctgctcccctccaaccatagctggtgggcttgcagcactggcctcaccccttgcctctccacctcagtttttaatcagactagagatttctgtatccaggtccagctgattcctcgcatctattactatcctgaagaagttttgttacaggcctatgacaattctcaccccaggactaaaagagaggctgtctcacttaccctagctgttttactggggttgggaatcacggcgggaataggtactggttcaactgccttaattaaaggacctatagacctccagcaaggcctgacaagcctccagatcgccatagatgctgacctccgggccctccaagactcagtcagcaagttagaggactcactgacttccctgtccgaggtagtgctccaaaataggagaggccttgacttgctgtttctaaaagaaggtggcctctgtgcggccctaaaggaagagtgctgtttttacatagaccactcaggtgcagtacgggactccatgaaaaaactcaaagaaaaactggataaaagacagttagagcgccagaaaagccaaaactggtatgaaggatggttcaataactccccttggttcactaccctgctatcaaccatcgctgggcccctattactcctccttctgttgctcatcctcgggccatgcatcatcaataagttagttcaattcatcaatgataggataagtgcagttaaaattctggtccttagacagaaatatcaggccctagagaacgaaggtaacctttaa

SEQ ID NO: 24 - protein, 685 aa, Gibbon ape leukemia virus
MVLLPGSMLLTSNLHHLRHQMSPGSWKRLIILLSCVFGGGGTSLQNKNPHQPMTLTWQVLSQTGDVVWDTKAVQPPWTWWPTLKPDVCALAASLESWDIPGTDVSSSKRVRPPDSDYTAAYKQITWGAIGCSYPRARTRMASSTFYVCPRDGRTLSEARRCGGLESLYCKEWDCETTGTGYWLSKSSKDLITVKWDQNSEWTQKFQQCHQTGWCNPLKIDFTDKGKLSKDWITGKTWGLRFYVSGHPGVQFTIRLKITNMPAVAVGPDLVLVEQGPPRTSLALPPPLPPREAPPPSLPDSNSTALATSAQTPTVRKTIVTLNTPPPTTGDRLFDLVQGAFLTLNATNPGATESCWLCLAMGPPYYEAIASSGEVAYSTDLDRCRWGTQGKLTLTEVSGHGLCIGKVPFTHQHLCNQTLSINSSGDHQYLLPSNHSWWACSTGLTPCLSTSVFNQTRDFCIQVQLIPRIYYYPEEVLLQAYDNSHPRTKREAVSLTLAVLLGLGITAGIGTGSTALIKGPIDLQQGLTSLQIAIDADLRALQDSVSKLEDSLTSLSEVVLQNRRGLDLLFLKEGGLCAALKEECCFYIDHSGAVRDSMKKLKEKLDKRQLERQKSQNWYEGWFNNSPWFTTLLSTIAGPLLLLLLLLILGPCIINKLVQFINDRISAVKILVLRQKYQALENEGNL